European Patent Specification EP 3 197 490 B1, published June 21, 2023. Title: METHODS AND COMPOSITIONS FOR INTRA-NASAL IMMUNIZATION WITH RECOMBINANT MVA ENCODING FLAGELLIN. Applicant: Bavarian Nordic A/S. The sequence listing filed with the application follows.

SEQUENCE LISTING (4 sequences)

SEQ ID NO: 1 - protein, 495 aa, Salmonella typhimurium [sequence omitted]

SEQ ID NO: 2 - DNA, 1488 bp, Salmonella typhimurium
atggcacaagtcattaatacaaacagcctgtcgctgttgacccagaataacctgaacaaatcccagtccgctctgggcaccgctatcgagcgtctgtcttccggtctgcgtatcaacagcgcgaaagacgatgcggcaggtcaggcgattgctaaccgttttaccgcgaacatcaaaggtctgactcaggcttcccgtaacgctaacgacggtatctccattgcgcagaccactgaaggcgcgctgaacgaaatcaacaacaacctgcagcgtgtgcgtgaactggcggttcagtctgctaacagcaccaactcccagtctgacctcgactccatccaggctgaaatcacccagcgcctgaacgaaatcgaccgtgtatccggccagactcagttcaacggcgtgaaagtcctggcgcaggacaacaccctgaccatccaggttggtgccaacgacggtgaaactatcgatatcgatctgaagcagatcaactctcagaccctgggtctggatacgctgaatgtgcaacaaaaatataaggtcagcgatacggctgcaactgttacaggatatgccgatactacgattgctttagacaatagtacttttaaagcctcggctactggtcttggtggtactgaccagaaaattgatggcgatttaaaatttgatgatacgactggaaaatattacgccaaagttaccgttacggggggaactggtaaagatggctattatgaagtttccgttgataagacgaacggtgaggtgactcttgctggcggtgcgacttccccgcttacaggtggactacctgcgacagcaactgaggatgtgaaaaatgtacaagttgcaaatgctgatttgacagaggctaaagccgcattgacagcagcaggtgttaccggcacagcatctgttgttaagatgtcttatactgataataacggtaaaactattgatggtggtttagcagttaaggtaggcgatgattactattctgcaactcaaaataaagatggttccataagtattaatactacgaaatacactgcagatgacggtacatccaaaactgcactaaacaaactgggtggcgcagacggcaaaaccgaagttgtttctattggtggtaaaacttacgctgcaagtaaagccgaaggtcacaactttaaagcacagcctgatctggcggaagcggctgctacaaccaccgaaaacccgctgcagaaaattgatgctgctttggcacaggttgacacgttacgttctgacctgggtgcggtacagaaccgtttcaactccgctattaccaacctgggcaacaccgtaaacaacctgacttctgcccgtagccgtatcgaagattccgactacgcgaccgaagtttccaacatgtctcgcgcgcagattctgcagcaggccggtacctccgttctggcgcaggcgaaccaggttccgcaaaacgtcctctctttactgcgttaa

SEQ ID NO: 3 - protein, 8 aa, Artificial
  Peptide
TSYKFESV

SEQ ID NO: 4 - protein, 8 aa, Artificial
  Peptide
SIINFEKL